European Patent Application EP 4 379 049 A1, published June 5, 2024. Title: Enzyme-containing composition, milk production method and fermented milk production method. Applicant: 合同酒精株式会社. Application JP, filed July 27, 2022. The sequence listing filed with the application follows.

SEQUENCE LISTING (4 sequences)

SEQ ID NO: 1 - protein, 741 aa, Streptomyces achromogenes
MTENHDAIVTDAKSEEGSGGCPVAHDRALHPTQGGGNRQWWPERLNVKILAKNPDVANPLDEDFDYAQAFQALDLAAVKRDIAEVLTTSQDWWPADFGNYGPLMIRMAWHSAGTYRISDGRGGAGAGQQRFAPLNSWPDNGNLDKARRLLWPVKKKYGQSISWADLLILTGNVALETMGFKTFGFGGGREDVWEPEEDVYWGPETTWLDDKRYTGDRELENPLGAVQMGLIYVNPEGPNGNPDPVAAARDIRETFRRMAMNDEETVALIAGGHTFGKTHGAGPADNVGPDPEAAGLEEQGLGWRNTYGTGKGGDAITSGLEVTWTTTPTQWSNGFFKNLFEYEYELEQSPAGAHQWVAKNAPEIVPDAHDPEKKHRPRMLTTDLALRFDPIYEPISRRFYENPEEFADAFARAWYKLTHRDMGPKSLYLGPEVPEETLLWQDPLPEREGELIDDADIAALKTKLLDSGLSVSQLVTTAWASASTFRASDKRGGANGARIRLAPQRGWEVNEPDQLAQVLRTLEGIQQEFNASSGAKKVSLADLIVLGGAAAVEKAAKEGGFAIEVPFTPGRVDAGEEHTDAESFEALEPTADGFRNYLGKGNRLPAEYLLLDRANLLSLSAPEMTALVGGLRVLGATYQQSQLGVLTKTPGVLTNDFFVNLLDMGTQWKATSEDQTTFEGRDASTGEVKWAGSRADLVFGSNSELRALAEVYASDDAKEKFVKDFVAAWNNVMNADRFDLV

SEQ ID NO: 2 - DNA, 2226 bp, Streptomyces achromogenes
  source 1..2226: mol_type = genomic DNA
atgactgagaaccacgacgcgatcgtcacagacgcgaagtcggaggaggggagcggcggctgccccgtcgcgcacgaccgggccctgcacccgacccagggcggtggcaaccgtcagtggtggccggagcggctcaatgtgaagatcctcgccaagaaccccgacgtggccaaccccctcgacgaggacttcgactacgcgcaggccttccaggccctggacctcgccgccgtgaagcgggacatcgccgaggtgctcaccacgtcgcaggactggtggcccgccgacttcggcaactacggccccctgatgatccgtatggcctggcacagcgcgggcacctaccgcatcagcgacggccgcggtggcgccggcgccggccagcagcgcttcgccccgctcaacagctggccggacaacggcaacctggacaaggcccgccgcctgctgtggccggtcaagaagaagtacggccagagcatctcctgggccgacctgctgatcctcaccggcaatgtcgccctggagacgatgggcttcaagaccttcggcttcggcggcggccgcgaggacgtctgggagccggaggaggacgtctactggggtcccgagaccacctggctggacgacaagcgctacaccggcgaccgcgagctggagaacccgctcggcgccgtccagatgggcctgatctacgtcaaccccgagggcccgaacggcaaccccgacccggtcgccgcggcccgcgacatccgtgagacgttccgccgcatggcgatgaacgacgaggagaccgtcgcgctgatcgccggcggccacaccttcggcaagacccacggcgccggtcccgccgacaacgtcggcccggacccggaggccgccggcctggaggagcagggcctcggctggcgcaacacctacggcaccggcaagggcggggacgccatcacctccggcctggaggtcacctggacgaccacgccgacccagtggagcaacgggttcttcaagaacctgttcgagtacgagtacgagctggagcagagcccggccggcgcccaccagtgggtcgccaagaacgccccggagatcgtccccgacgcgcacgacccggagaagaagcaccgcccgcggatgctcaccaccgacctggcgctgcgcttcgacccgatctacgagcccatctcccgccggttctacgagaacccggaggaattcgcggacgccttcgcccgcgcctggtacaagctcacccaccgcgacatgggcccgaagtcgctgtacctcggccccgaggtcccggaggagacgctgctctggcaggacccgctgcccgagcgcgagggcgagctgatcgacgacgccgacatcgccgccctgaagaccaagctgctcgactcgggtctgtccgtgtcccagctggtcaccaccgcgtgggcgtccgcgtccacgttccgcgccagcgacaagcgcggcggcgccaacggcgcccgcatccgcctcgccccgcagcgcggctgggaggtcaacgagcccgaccagctcgcccaggtgctgcgcaccctggagggcatccagcaggagttcaacgcctcctccggcgccaagaaggtctccctggccgacctcatcgtcctcggcggtgccgccgccgtggagaaggccgccaaggagggcggcttcgcgatcgaggtgcccttcaccccgggccgggtggacgccggcgaggagcacaccgacgccgagtccttcgaggcgctggagccgaccgcggacggcttccgcaactacctcggcaagggcaaccgcctgcccgccgagtacctgctgctcgaccgggccaacctgctgagcctgagtgcccccgagatgaccgcgctcgtcggcggtctgcgcgtcctcggcgccacctaccagcagtcgcagctcggcgtgctcaccaagacgcccggcgtcctcaccaacgacttcttcgtcaacctgctcgacatgggcacgcagtggaaggcgacctcggaggaccagaccaccttcgagggccgggacgcgagcaccggcgaggtgaagtgggccggcagccgggccgacctcgtcttcggctccaactccgagctgcgcgccctcgccgaggtgtacgcgagcgacgacgccaaggagaagttcgtgaaggacttcgtcgccgcgtggaacaatgtcatgaacgcggaccgcttcgacctcgtctga

SEQ ID NO: 3 - DNA, 29 bp, synthetic construct
  source 1..29: mol_type = other DNA
tagaattccatatgactgagaaccacgac

SEQ ID NO: 4 - DNA, 46 bp, synthetic construct
  source 1..46: mol_type = other DNA
ccccaagctttcaatgatgatgatgatgatggacgaggtcgaagcg